European Patent Application EP 4 349 990 A1, published April 10, 2024. Title: Artificial polynucleotides for expressing proteins. Applicant: CERTEST BIOTEC, S.L. The sequence listing filed with the application follows.

SEQUENCE LISTING (39 sequences)

SEQ ID NO: 1 - RNA, 12 nt, synthetic construct
  source 1..12: mol_type = other RNA
gccnccgccncc

SEQ ID NO: 2 - RNA, 12 nt, synthetic construct
  source 1..12: mol_type = other RNA
gccrccgccrcc

SEQ ID NO: 3 - RNA, 12 nt, synthetic construct
  source 1..12: mol_type = other RNA
gccaccgccacc

SEQ ID NO: 4 - RNA, 12 nt, synthetic construct
  source 1..12: mol_type = other RNA
gccaccgccgcc

SEQ ID NO: 5 - RNA, 12 nt, synthetic construct
  source 1..12: mol_type = other RNA
gccgccgccacc

SEQ ID NO: 6 - RNA, 12 nt, synthetic construct
  source 1..12: mol_type = other RNA
gccgccgccgcc

SEQ ID NO: 7 - RNA, 58 nt, Homo sapiens
  source 1..58: mol_type = other RNA
aggcacagacaccaaggacagagacgctggctaggccgccctccccactgttaccaac

SEQ ID NO: 8 - RNA, 64 nt, synthetic construct
  source 1..64: mol_type = other RNA
aggcacagacaccaaggacagagacgctggctaggccgccctccccactgttaccaacgccacc

SEQ ID NO: 9 - RNA, 70 nt, synthetic construct
  source 1..70: mol_type = other RNA
aggcacagacaccaaggacagagacgctggctaggccgccctccccactgttaccaacgccaccgccacc

SEQ ID NO: 10 - RNA, 50 nt, Homo sapiens
  source 1..50: mol_type = other RNA
acatttgcttctgacacaactgtgttcactagcaacctcaaacagacacc

SEQ ID NO: 11 - RNA, 56 nt, synthetic construct
  source 1..56: mol_type = other RNA
acatttgcttctgacacaactgtgttcactagcaacctcaaacagacaccgccacc

SEQ ID NO: 12 - RNA, 62 nt, synthetic construct
  source 1..62: mol_type = other RNA
acatttgcttctgacacaactgtgttcactagcaacctcaaacagacaccgccaccgccacc

SEQ ID NO: 13 - RNA, 81 nt, Homo sapiens
  source 1..81: mol_type = other RNA
tagaaggcagtcttgtgggtgcctcctcccccagccgcaactcaggtctgcagctgggtcctgcctccttccgagtgggcc

SEQ ID NO: 14 - RNA, 87 nt, synthetic construct
  source 1..87: mol_type = other RNA
tagaaggcagtcttgtgggtgcctcctcccccagccgcaactcaggtctgcagctgggtcctgcctccttccgagtgggccgccacc

SEQ ID NO: 15 - RNA, 93 nt, synthetic construct
  source 1..93: mol_type = other RNA
tagaaggcagtcttgtgggtgcctcctcccccagccgcaactcaggtctgcagctgggtcctgcctccttccgagtgggccgccaccgccacc

SEQ ID NO: 16 - RNA, 54 nt, synthetic construct
  source 1..54: mol_type = other RNA
aaataagagagaaaagaagagtaagaagaaatataagaccccggcgccgccacc

SEQ ID NO: 17 - RNA, 44 nt, synthetic construct
  source 1..44: mol_type = other RNA
aaataagagagaaaagaagagtaagaagaaatataagagccacc

SEQ ID NO: 18 - RNA, 132 nt, Homo sapiens
  source 1..132: mol_type = other RNA
gctcgctttcttgctgtccaatttctattaaaggttcctttgttccctaagtccaactactaaactgggggatattatgaagggccttgagcatctggattctgcctaataaaaaacatttattttcattgc

SEQ ID NO: 19 - RNA, 264 nt, synthetic construct
  source 1..264: mol_type = other RNA
gctcgctttcttgctgtccaatttctattaaaggttcctttgttccctaagtccaactactaaactgggggatattatgaagggccttgagcatctggattctgcctaataaaaaacatttattttcattgcgctcgctttcttgctgtccaatttctattaaaggttcctttgttccctaagtccaactactaaactgggggatattatgaagggccttgagcatctggattctgcctaataaaaaacatttattttcattgc

SEQ ID NO: 20 - RNA, 153 nt, Homo sapiens
  source 1..153: mol_type = other RNA
gggcagggctctacctcccctgcgtcacactgtgtgaggctgtgtctctgccatccaaaagggggccccttgagaatggtgatccacccagttacaggggcatttagggagcagatgactgagaacattaaaaaagaacttaaatgacacagc

SEQ ID NO: 21 - RNA, 306 nt, synthetic construct
  source 1..306: mol_type = other RNA
gggcagggctctacctcccctgcgtcacactgtgtgaggctgtgtctctgccatccaaaagggggccccttgagaatggtgatccacccagttacaggggcatttagggagcagatgactgagaacattaaaaaagaacttaaatgacacagcgggcagggctctacctcccctgcgtcacactgtgtgaggctgtgtctctgccatccaaaagggggccccttgagaatggtgatccacccagttacaggggcatttagggagcagatgactgagaacattaaaaaagaacttaaatgacacagc

SEQ ID NO: 22 - RNA, 113 nt, Homo sapiens
  source 1..113: mol_type = other RNA
agtgtccagaccattgtcttccaaccccagctggcctctagaacacccactggccagtcctagagctcctgtccctacccactctttgctacaataaatgctgaatgaatcca

SEQ ID NO: 23 - RNA, 226 nt, synthetic construct
  source 1..226: mol_type = other RNA
agtgtccagaccattgtcttccaaccccagctggcctctagaacacccactggccagtcctagagctcctgtccctacccactctttgctacaataaatgctgaatgaatccaagtgtccagaccattgtcttccaaccccagctggcctctagaacacccactggccagtcctagagctcctgtccctacccactctttgctacaataaatgctgaatgaatcca

SEQ ID NO: 24 - RNA, 110 nt, synthetic construct
  source 1..110: mol_type = other RNA
gctggagcctcggtggcctagcttcttgccccttgggcctccccccagcccctcctccccttcctgcacccgtacccccgtggtctttgaataaagtctgagtgggcggc

SEQ ID NO: 25 - RNA, 109 nt, Homo sapiens
  source 1..109: mol_type = other RNA
gctggagcctcggtggccatgcttcttgccccttgggcctccccccagcccctcctccccttcctgcacccgtacccccgtggtctttgaataaagtctgagtgggcgg

SEQ ID NO: 26 - RNA, 101 nt, Mus musculus
  source 1..101: mol_type = other RNA
ttaattaagctgccttctgcggggcttgccttctggccatgcccttcttctctcccttgcacctgtacctcttggtctttgaataaagcctgagtaggaag

SEQ ID NO: 27 - RNA, 2082 nt, synthetic construct
  source 1..2082: mol_type = other RNA
aggaggcacagacaccaaggacagagacgctggctaggccgccctccccactgttaccaacatggaggacgccaagaacatcaagaagggccccgcccccttctaccccctggaggacggcaccgccggcgagcagctgcacaaggccatgaagaggtacgccctggtgcccggcaccatcgccttcaccgacgcccacatcgaggtggacatcacctacgccgagtacttcgagatgagcgtgaggctggccgaggccatgaagaggtacggcctgaacaccaaccacaggatcgtggtgtgcagcgagaacagcctgcagttcttcatgcccgtgctgggcgccctgttcatcggcgtggccgtggcccccgccaacgacatctacaacgagagggagctgctgaacagcatgggcatcagccagcccaccgtggtgttcgtgagcaagaagggcctgcagaagatcctgaacgtgcagaagaagctgcccatcatccagaagatcatcatcatggacagcaagaccgactaccagggcttccagagcatgtacaccttcgtgaccagccacctgccccccggcttcaacgagtacgacttcgtgcccgagagcttcgacagggacaagaccatcgccctgatcatgaacagcagcggcagcaccggcctgcccaagggcgtggccctgccccacaggaccgcctgcgtgaggttcagccacgccagggaccccatcttcggcaaccagatcatccccgacaccgccatcctgagcgtggtgcccttccaccacggcttcggcatgttcaccaccctgggctacctgatctgcggcttcagggtggtgctgatgtacaggttcgaggaggagctgttcctgaggagcctgcaggactacaagatccagagcgccctgctggtgcccaccctgttcagcttcttcgccaagagcaccctgatcgacaagtacgacctgagcaacctgcacgagatcgccagcggcggcgcccccctgagcaaggaggtgggcgaggccgtggccaagaggttccacctgcccggcatcaggcagggctacggcctgaccgagaccaccagcgccatcctgatcacccccgagggcgacgacaagcccggcgccgtgggcaaggtggtgcccttcttcgaggccaaggtggtggacctggacaccggcaagaccctgggcgtgaaccagaggggcgagctgtgcgtgaggggccccatgatcatgagcggctacgtgaacaaccccgaggccaccaacgccctgatcgacaaggacggctggctgcacagcggcgacatcgcctactgggacgaggacgagcacttcttcatcgtggacaggctgaagagtctgatcaagtacaagggctaccaggtggcccccgccgagctggagagcatcctgctgcagcaccccaacatcttcgacgccggcgtggccggcctgcccgacgacgacgccggcgagctgcccgccgccgtggtggtgctggagcacggcaagaccatgaccgagaaggagatcgtggactacgtggccagccaggtgaccaccgccaagaagctgaggggcggcgtggtgttcgtggacgaggtgcccaagggcctgaccggcaagctggacgccaggaagatcagggagatcctgatcaaggccaagaagggcggcaagatcgccgtgtgatgagctcgctttcttgctgtccaatttctattaaaggttcctttgttccctaagtccaactactaaactgggggatattatgaagggccttgagcatctggattctgcctaataaaaaacatttattttcattgcgctcgctttcttgctgtccaatttctattaaaggttcctttgttccctaagtccaactactaaactgggggatattatgaagggccttgagcatctggattctgcctaataaaaaacatttattttcattgcaaaaaaaaaaaaaaaaaaaaaaaaaaaaaagaaaaaaaaaaaaaaaaaaaaaaaaaaaaaaaaaaaaaaaaaaaaaaaaaaaaaaaaaaaaaaaaaaaaaa

SEQ ID NO: 28 - RNA, 2088 nt, synthetic construct
  source 1..2088: mol_type = other RNA
aggaggcacagacaccaaggacagagacgctggctaggccgccctccccactgttaccaacgccaccatggaggacgccaagaacatcaagaagggccccgcccccttctaccccctggaggacggcaccgccggcgagcagctgcacaaggccatgaagaggtacgccctggtgcccggcaccatcgccttcaccgacgcccacatcgaggtggacatcacctacgccgagtacttcgagatgagcgtgaggctggccgaggccatgaagaggtacggcctgaacaccaaccacaggatcgtggtgtgcagcgagaacagcctgcagttcttcatgcccgtgctgggcgccctgttcatcggcgtggccgtggcccccgccaacgacatctacaacgagagggagctgctgaacagcatgggcatcagccagcccaccgtggtgttcgtgagcaagaagggcctgcagaagatcctgaacgtgcagaagaagctgcccatcatccagaagatcatcatcatggacagcaagaccgactaccagggcttccagagcatgtacaccttcgtgaccagccacctgccccccggcttcaacgagtacgacttcgtgcccgagagcttcgacagggacaagaccatcgccctgatcatgaacagcagcggcagcaccggcctgcccaagggcgtggccctgccccacaggaccgcctgcgtgaggttcagccacgccagggaccccatcttcggcaaccagatcatccccgacaccgccatcctgagcgtggtgcccttccaccacggcttcggcatgttcaccaccctgggctacctgatctgcggcttcagggtggtgctgatgtacaggttcgaggaggagctgttcctgaggagcctgcaggactacaagatccagagcgccctgctggtgcccaccctgttcagcttcttcgccaagagcaccctgatcgacaagtacgacctgagcaacctgcacgagatcgccagcggcggcgcccccctgagcaaggaggtgggcgaggccgtggccaagaggttccacctgcccggcatcaggcagggctacggcctgaccgagaccaccagcgccatcctgatcacccccgagggcgacgacaagcccggcgccgtgggcaaggtggtgcccttcttcgaggccaaggtggtggacctggacaccggcaagaccctgggcgtgaaccagaggggcgagctgtgcgtgaggggccccatgatcatgagcggctacgtgaacaaccccgaggccaccaacgccctgatcgacaaggacggctggctgcacagcggcgacatcgcctactgggacgaggacgagcacttcttcatcgtggacaggctgaagagtctgatcaagtacaagggctaccaggtggcccccgccgagctggagagcatcctgctgcagcaccccaacatcttcgacgccggcgtggccggcctgcccgacgacgacgccggcgagctgcccgccgccgtggtggtgctggagcacggcaagaccatgaccgagaaggagatcgtggactacgtggccagccaggtgaccaccgccaagaagctgaggggcggcgtggtgttcgtggacgaggtgcccaagggcctgaccggcaagctggacgccaggaagatcagggagatcctgatcaaggccaagaagggcggcaagatcgccgtgtgatgagctcgctttcttgctgtccaatttctattaaaggttcctttgttccctaagtccaactactaaactgggggatattatgaagggccttgagcatctggattctgcctaataaaaaacatttattttcattgcgctcgctttcttgctgtccaatttctattaaaggttcctttgttccctaagtccaactactaaactgggggatattatgaagggccttgagcatctggattctgcctaataaaaaacatttattttcattgcaaaaaaaaaaaaaaaaaaaaaaaaaaaaaagaaaaaaaaaaaaaaaaaaaaaaaaaaaaaaaaaaaaaaaaaaaaaaaaaaaaaaaaaaaaaaaaaaaaaa

SEQ ID NO: 29 - RNA, 2094 nt, synthetic construct
  source 1..2094: mol_type = other RNA
aggaggcacagacaccaaggacagagacgctggctaggccgccctccccactgttaccaacgccaccgccaccatggaggacgccaagaacatcaagaagggccccgcccccttctaccccctggaggacggcaccgccggcgagcagctgcacaaggccatgaagaggtacgccctggtgcccggcaccatcgccttcaccgacgcccacatcgaggtggacatcacctacgccgagtacttcgagatgagcgtgaggctggccgaggccatgaagaggtacggcctgaacaccaaccacaggatcgtggtgtgcagcgagaacagcctgcagttcttcatgcccgtgctgggcgccctgttcatcggcgtggccgtggcccccgccaacgacatctacaacgagagggagctgctgaacagcatgggcatcagccagcccaccgtggtgttcgtgagcaagaagggcctgcagaagatcctgaacgtgcagaagaagctgcccatcatccagaagatcatcatcatggacagcaagaccgactaccagggcttccagagcatgtacaccttcgtgaccagccacctgccccccggcttcaacgagtacgacttcgtgcccgagagcttcgacagggacaagaccatcgccctgatcatgaacagcagcggcagcaccggcctgcccaagggcgtggccctgccccacaggaccgcctgcgtgaggttcagccacgccagggaccccatcttcggcaaccagatcatccccgacaccgccatcctgagcgtggtgcccttccaccacggcttcggcatgttcaccaccctgggctacctgatctgcggcttcagggtggtgctgatgtacaggttcgaggaggagctgttcctgaggagcctgcaggactacaagatccagagcgccctgctggtgcccaccctgttcagcttcttcgccaagagcaccctgatcgacaagtacgacctgagcaacctgcacgagatcgccagcggcggcgcccccctgagcaaggaggtgggcgaggccgtggccaagaggttccacctgcccggcatcaggcagggctacggcctgaccgagaccaccagcgccatcctgatcacccccgagggcgacgacaagcccggcgccgtgggcaaggtggtgcccttcttcgaggccaaggtggtggacctggacaccggcaagaccctgggcgtgaaccagaggggcgagctgtgcgtgaggggccccatgatcatgagcggctacgtgaacaaccccgaggccaccaacgccctgatcgacaaggacggctggctgcacagcggcgacatcgcctactgggacgaggacgagcacttcttcatcgtggacaggctgaagagtctgatcaagtacaagggctaccaggtggcccccgccgagctggagagcatcctgctgcagcaccccaacatcttcgacgccggcgtggccggcctgcccgacgacgacgccggcgagctgcccgccgccgtggtggtgctggagcacggcaagaccatgaccgagaaggagatcgtggactacgtggccagccaggtgaccaccgccaagaagctgaggggcggcgtggtgttcgtggacgaggtgcccaagggcctgaccggcaagctggacgccaggaagatcagggagatcctgatcaaggccaagaagggcggcaagatcgccgtgtgatgagctcgctttcttgctgtccaatttctattaaaggttcctttgttccctaagtccaactactaaactgggggatattatgaagggccttgagcatctggattctgcctaataaaaaacatttattttcattgcgctcgctttcttgctgtccaatttctattaaaggttcctttgttccctaagtccaactactaaactgggggatattatgaagggccttgagcatctggattctgcctaataaaaaacatttattttcattgcaaaaaaaaaaaaaaaaaaaaaaaaaaaaaagaaaaaaaaaaaaaaaaaaaaaaaaaaaaaaaaaaaaaaaaaaaaaaaaaaaaaaaaaaaaaaaaaaaaaa

SEQ ID NO: 30 - RNA, 1936 nt, synthetic construct
  source 1..1936: mol_type = other RNA
aggaaataagagagaaaagaagagtaagaagaaatataagaccccggcgccgccaccatggaggacgccaagaacatcaagaagggccccgcccccttctaccccctggaggacggcaccgccggcgagcagctgcacaaggccatgaagaggtacgccctggtgcccggcaccatcgccttcaccgacgcccacatcgaggtggacatcacctacgccgagtacttcgagatgagcgtgaggctggccgaggccatgaagaggtacggcctgaacaccaaccacaggatcgtggtgtgcagcgagaacagcctgcagttcttcatgcccgtgctgggcgccctgttcatcggcgtggccgtggcccccgccaacgacatctacaacgagagggagctgctgaacagcatgggcatcagccagcccaccgtggtgttcgtgagcaagaagggcctgcagaagatcctgaacgtgcagaagaagctgcccatcatccagaagatcatcatcatggacagcaagaccgactaccagggcttccagagcatgtacaccttcgtgaccagccacctgccccccggcttcaacgagtacgacttcgtgcccgagagcttcgacagggacaagaccatcgccctgatcatgaacagcagcggcagcaccggcctgcccaagggcgtggccctgccccacaggaccgcctgcgtgaggttcagccacgccagggaccccatcttcggcaaccagatcatccccgacaccgccatcctgagcgtggtgcccttccaccacggcttcggcatgttcaccaccctgggctacctgatctgcggcttcagggtggtgctgatgtacaggttcgaggaggagctgttcctgaggagcctgcaggactacaagatccagagcgccctgctggtgcccaccctgttcagcttcttcgccaagagcaccctgatcgacaagtacgacctgagcaacctgcacgagatcgccagcggcggcgcccccctgagcaaggaggtgggcgaggccgtggccaagaggttccacctgcccggcatcaggcagggctacggcctgaccgagaccaccagcgccatcctgatcacccccgagggcgacgacaagcccggcgccgtgggcaaggtggtgcccttcttcgaggccaaggtggtggacctggacaccggcaagaccctgggcgtgaaccagaggggcgagctgtgcgtgaggggccccatgatcatgagcggctacgtgaacaaccccgaggccaccaacgccctgatcgacaaggacggctggctgcacagcggcgacatcgcctactgggacgaggacgagcacttcttcatcgtggacaggctgaagagtctgatcaagtacaagggctaccaggtggcccccgccgagctggagagcatcctgctgcagcaccccaacatcttcgacgccggcgtggccggcctgcccgacgacgacgccggcgagctgcccgccgccgtggtggtgctggagcacggcaagaccatgaccgagaaggagatcgtggactacgtggccagccaggtgaccaccgccaagaagctgaggggcggcgtggtgttcgtggacgaggtgcccaagggcctgaccggcaagctggacgccaggaagatcagggagatcctgatcaaggccaagaagggcggcaagatcgccgtgtgataataggctggagcctcggtggcctagcttcttgccccttgggcctccccccagcccctcctccccttcctgcacccgtacccccgtggtctttgaataaagtctgagtgggcggcaaaaaaaaaaaaaaaaaaaaaaaaaaaaaagcatatgactaaaaaaaaaaaaaaaaaaaaaaaaaaaaaaaaaaaaaaaaaaaaaaaaaaaaaaaaaaaaaaaaaaaaaa

SEQ ID NO: 31 - RNA, 1915 nt, synthetic construct
  source 1..1915: mol_type = other RNA
aggaaataagagagaaaagaagagtaagaagaaatataagagccaccatggaagacgccaagaacattaagaaggggccggccccgttctacccgttggaagacgggaccgccggggaacagttgcacaaggccatgaagagatacgccttggtgccggggaccattgccttcaccgacgcccacattgaagtggacattacctacgccgaatacttcgaaatgtcggtgagattggccgaagccatgaagagatacgggttgaacaccaaccacagaattgtggtgtgctcggaaaactcgttgcagttcttcatgccggtgttgggggccttgttcattggggtggccgtggccccggccaacgacatttacaacgaaagagaattgttgaactcgatggggatttcgcagccgaccgtggtgttcgtgtcgaagaaggggttgcagaagattttgaacgtgcagaagaagttgccgattattcagaagattattattatggactcgaagaccgactaccaggggttccagtcgatgtacaccttcgtgacctcgcacttgccgccggggttcaacgaatacgacttcgtgccggaatcgttcgacagagacaagaccattgccttgattatgaactcgtcggggtcgaccgggttgccgaagggggtggccttgccgcacagaaccgcctgcgtgagattctcgcacgccagagacccgattttcgggaaccagattattccggacaccgccattttgtcggtggtgccgttccaccacgggttcgggatgttcaccaccttggggtacttgatttgcgggttcagagtggtgttgatgtacagattcgaagaagaattgttcttgagatcgttgcaggactacaagattcagtcggccttgttggtgccgaccttgttctcgttcttcgccaagtcgaccttgattgacaagtacgacttgtcgaacttgcacgaaattgcctcggggggggccccgttgtcgaaggaagtgggggaagccgtggccaagagattccacttgccggggattagacaggggtacgggttgaccgaaaccacctcggccattttgattaccccggaaggggacgacaagccgggggccgtggggaaggtggtgccgttcttcgaagccaaggtggtggacttggacaccgggaagaccttgggggtgaaccagagaggggaattgtgcgtgagagggccgatgattatgtcggggtacgtgaacaacccggaagccaccaacgccttgattgacaaggacgggtggttgcactcgggggacattgcctactgggacgaagacgaacacttcttcattgtggacagattgaagtcgttgattaagtacaaggggtaccaggtggccccggccgaattggaatcgattttgttgcagcacccgaacattttcgacgccggggtggccgggttgccggacgacgacgccggggaattgccggccgccgtggtggtgttggaacacgggaagaccatgaccgaaaaggaaattgtggactacgtggcctcgcaggtgaccaccgccaagaagttgagagggggggtggtgttcgtggacgaagtgccgaaggggttgaccgggaagttggacgccagaaagattagagaaattttgattaaggccaagaagggggggaagattgccgtgtgataataggctggagcctcggtggccatgcttcttgccccttgggcctccccccagcccctcctccccttcctgcacccgtacccccgtggtctttgaataaagtctgagtgggcggaaaaaaaaaaaaaaaaaaaaaaaaaaaaaaaaaaaaaaaaaaaaaaaaaaaaaaaaaaaaaaaaaaaaaaaaaaaaaaaaaaaaaaaaaaaaaaaaaaaa

SEQ ID NO: 32 - RNA, 1903 nt, synthetic construct
  source 1..1903: mol_type = other RNA
aggaaataagagagaaaagaagagtaagaagaaatataagagccaccatggaggacgccaagaacatcaagaagggccccgcccccttctaccccctggaggacggcaccgccggcgagcagctgcacaaggccatgaagcggtacgccctggtgcccggcaccatcgccttcaccgacgcccacatcgaggtggacatcacctacgccgagtacttcgagatgagcgtgcggctggccgaggccatgaagcggtacggcctgaacaccaaccaccggatcgtggtgtgcagcgagaacagcctgcagttcttcatgcccgtgctgggcgccctgttcatcggcgtggccgtggcccccgccaacgacatctacaacgagcgggagctgctgaacagcatgggcatcagccagcccaccgtggtgttcgtgagcaagaagggcctgcagaagatcctgaacgtgcagaagaagctgcccatcatccagaagatcatcatcatggacagcaagaccgactaccagggcttccagagcatgtacaccttcgtgaccagccacctgccccccggcttcaacgagtacgacttcgtgcccgagagcttcgaccgggacaagaccatcgccctgatcatgaacagcagcggcagcaccggcctgcccaagggcgtggccctgccccaccggaccgcctgcgtgcggttcagccacgcccgggaccccatcttcggcaaccagatcatccccgacaccgccatcctgagcgtggtgcccttccaccacggcttcggcatgttcaccaccctgggctacctgatctgcggcttccgggtggtgctgatgtaccggttcgaggaggagctgttcctgcggagcctgcaggactacaagatccagagcgccctgctggtgcccaccctgttcagcttcttcgccaagagcaccctgatcgacaagtacgacctgagcaacctgcacgagatcgccagcggcggcgcccccctgagcaaggaggtgggcgaggccgtggccaagcggttccacctgcccggcatccggcagggctacggcctgaccgagaccaccagcgccatcctgatcacccccgagggcgacgacaagcccggcgccgtgggcaaggtggtgcccttcttcgaggccaaggtggtggacctggacaccggcaagaccctgggcgtgaaccagcggggcgagctgtgcgtgcggggccccatgatcatgagcggctacgtgaacaaccccgaggccaccaacgccctgatcgacaaggacggctggctgcacagcggcgacatcgcctactgggacgaggacgagcacttcttcatcgtggaccggctgaagagcctgatcaagtacaagggctaccaggtggcccccgccgagctggagagcatcctgctgcagcaccccaacatcttcgacgccggcgtggccggcctgcccgacgacgacgccggcgagctgcccgccgccgtggtggtgctggagcacggcaagaccatgaccgagaaggagatcgtggactacgtggccagccaggtgaccaccgccaagaagctgcggggcggcgtggtgttcgtggacgaggtgcccaagggcctgaccggcaagctggacgcccggaagatccgggagatcctgatcaaggccaagaagggcggcaagatcgccgtgtgattaattaagctgccttctgcggggcttgccttctggccatgcccttcttctctcccttgcacctgtacctcttggtctttgaataaagcctgagtaggaagaaaaaaaaaaaaaaaaaaaaaaaaaaaaaaaaaaaaaaaaaaaaaaaaaaaaaaaaaaaaaaaaaaaaaaaaaaaaaaaaaaaaaaaaaaaaaaaaaaaaaa

SEQ ID NO: 33 - DNA, 3931 bp, synthetic construct
  source 1..3931: mol_type = other DNA
tcgcgcgtttcggtgatgacggtgaaaacctctgacacatgcagctcccggacgtcattgtcgattaatacgactcactataaggaggcacagacaccaaggacagagacgctggctaggccgccctccccactgttaccaacatggaggacgccaagaacatcaagaagggccccgcccccttctaccccctggaggacggcaccgccggcgagcagctgcacaaggccatgaagaggtacgccctggtgcccggcaccatcgccttcaccgacgcccacatcgaggtggacatcacctacgccgagtacttcgagatgagcgtgaggctggccgaggccatgaagaggtacggcctgaacaccaaccacaggatcgtggtgtgcagcgagaacagcctgcagttcttcatgcccgtgctgggcgccctgttcatcggcgtggccgtggcccccgccaacgacatctacaacgagagggagctgctgaacagcatgggcatcagccagcccaccgtggtgttcgtgagcaagaagggcctgcagaagatcctgaacgtgcagaagaagctgcccatcatccagaagatcatcatcatggacagcaagaccgactaccagggcttccagagcatgtacaccttcgtgaccagccacctgccccccggcttcaacgagtacgacttcgtgcccgagagcttcgacagggacaagaccatcgccctgatcatgaacagcagcggcagcaccggcctgcccaagggcgtggccctgccccacaggaccgcctgcgtgaggttcagccacgccagggaccccatcttcggcaaccagatcatccccgacaccgccatcctgagcgtggtgcccttccaccacggcttcggcatgttcaccaccctgggctacctgatctgcggcttcagggtggtgctgatgtacaggttcgaggaggagctgttcctgaggagcctgcaggactacaagatccagagcgccctgctggtgcccaccctgttcagcttcttcgccaagagcaccctgatcgacaagtacgacctgagcaacctgcacgagatcgccagcggcggcgcccccctgagcaaggaggtgggcgaggccgtggccaagaggttccacctgcccggcatcaggcagggctacggcctgaccgagaccaccagcgccatcctgatcacccccgagggcgacgacaagcccggcgccgtgggcaaggtggtgcccttcttcgaggccaaggtggtggacctggacaccggcaagaccctgggcgtgaaccagaggggcgagctgtgcgtgaggggccccatgatcatgagcggctacgtgaacaaccccgaggccaccaacgccctgatcgacaaggacggctggctgcacagcggcgacatcgcctactgggacgaggacgagcacttcttcatcgtggacaggctgaagagtctgatcaagtacaagggctaccaggtggcccccgccgagctggagagcatcctgctgcagcaccccaacatcttcgacgccggcgtggccggcctgcccgacgacgacgccggcgagctgcccgccgccgtggtggtgctggagcacggcaagaccatgaccgagaaggagatcgtggactacgtggccagccaggtgaccaccgccaagaagctgaggggcggcgtggtgttcgtggacgaggtgcccaagggcctgaccggcaagctggacgccaggaagatcagggagatcctgatcaaggccaagaagggcggcaagatcgccgtgtgatgagctcgctttcttgctgtccaatttctattaaaggttcctttgttccctaagtccaactactaaactgggggatattatgaagggccttgagcatctggattctgcctaataaaaaacatttattttcattgcgctcgctttcttgctgtccaatttctattaaaggttcctttgttccctaagtccaactactaaactgggggatattatgaagggccttgagcatctggattctgcctaataaaaaacatttattttcattgcaaaaaaaaaaaaaaaaaaaaaaaaaaaaaagaaaaaaaaaaaaaaaaaaaaaaaaaaaaaaaaaaaaaaaaaaaaaaaaaaaaaaaaaaaaaaaaaaaaaacgaagagcatcattgtcacatgtgagcaaaaggccagcaaaaggccaggaaccgtaaaaaggccgcgttgctggcgtttttccataggctccgcccccctgacgagcatcacaaaaatcgacgctcaagtcagaggtggcgaaacccgacaggactataaagataccaggcgtttccccctggaagctccctcgtgcgctctcctgttccgaccctgccgcttaccggatacctgtccgcctttctcccttcgggaagcgtggcgctttctcatagctcacgctgtaggtatctcagttcggtgtaggtcgttcgctccaagctgggctgtgtgcacgaaccccccgttcagcccgaccgctgcgccttatccggtaactatcgtcttgagtccaacccggtaagacacgacttatcgccactggcagcagccactggtaacaggattagcagagcgaggtatgtaggcggtgctacagagttcttgaagtggtggcctaactacggctacactagaagaacagtatttggtatctgcgctctgctgaagccagttaccttcggaaaaagagttggtagctcttgatccggcaaacaaaccaccgctggtagcggtggtttttttgtttgcaagcagcagattacgcgcagaaaaaaaggatctcaagaagatcctttgatcttttctacggggtctgacgctcagtggaacgaaaactcacgttaagggattttggtcatgagattatcaaaaaggatcttcacctagatccttttaaattaaaaatgaagttttaaatcaagcccaatctgaataatgttacaaccaattaaccaattctgattagaaaaactcatcgagcatcaaatgaaactgcaatttattcatatcaggattatcaataccatatttttgaaaaagccgtttctgtaatgaaggagaaaactcaccgaggcagttccataggatggcaagatcctggtatcggtctgcgattccgactcgtccaacatcaatacaacctattaatttcccctcgtcaaaaataaggttatcaagtgagaaatcaccatgagtgacgactgaatccggtgagaatggcaaaagtttatgcatttctttccagacttgttcaacaggccagccattacgctcgtcatcaaaatcactcgcatcaaccaaaccgttattcattcgtgattgcgcctgagcgagacgaaatacgcgatcgctgttaaaaggacaattacaaacaggaatcgaatgcaaccggcgcaggaacactgccagcgcatcaacaatattttcacctgaatcaggatattcttctaatacctggaatgctgtttttccggggatcgcagtggtgagtaaccatgcatcatcaggagtacggataaaatgcttgatggtcggaagaggcataaattccgtcagccagtttagtctgaccatctcatctgtaacatcattggcaacgctacctttgccatgtttcagaaacaactctggcgcatcgggcttcccatacaagcgatagattgtcgcacctgattgcccgacattatcgcgagcccatttatacccatataaatcagcatccatgttggaatttaatcgcggcctcgacgtttcccgttgaatatggctcataacaccccttgtattactgtttatgtaagcagacagttttattgttcatgatgatatatttttatcttgtgcaatgtaacatcagagattttgagacacgggccagagctgca

SEQ ID NO: 34 - DNA, 3937 bp, synthetic construct
  source 1..3937: mol_type = other DNA
tcgcgcgtttcggtgatgacggtgaaaacctctgacacatgcagctcccggacgtcattgtcgattaatacgactcactataaggaggcacagacaccaaggacagagacgctggctaggccgccctccccactgttaccaacgccaccatggaggacgccaagaacatcaagaagggccccgcccccttctaccccctggaggacggcaccgccggcgagcagctgcacaaggccatgaagaggtacgccctggtgcccggcaccatcgccttcaccgacgcccacatcgaggtggacatcacctacgccgagtacttcgagatgagcgtgaggctggccgaggccatgaagaggtacggcctgaacaccaaccacaggatcgtggtgtgcagcgagaacagcctgcagttcttcatgcccgtgctgggcgccctgttcatcggcgtggccgtggcccccgccaacgacatctacaacgagagggagctgctgaacagcatgggcatcagccagcccaccgtggtgttcgtgagcaagaagggcctgcagaagatcctgaacgtgcagaagaagctgcccatcatccagaagatcatcatcatggacagcaagaccgactaccagggcttccagagcatgtacaccttcgtgaccagccacctgccccccggcttcaacgagtacgacttcgtgcccgagagcttcgacagggacaagaccatcgccctgatcatgaacagcagcggcagcaccggcctgcccaagggcgtggccctgccccacaggaccgcctgcgtgaggttcagccacgccagggaccccatcttcggcaaccagatcatccccgacaccgccatcctgagcgtggtgcccttccaccacggcttcggcatgttcaccaccctgggctacctgatctgcggcttcagggtggtgctgatgtacaggttcgaggaggagctgttcctgaggagcctgcaggactacaagatccagagcgccctgctggtgcccaccctgttcagcttcttcgccaagagcaccctgatcgacaagtacgacctgagcaacctgcacgagatcgccagcggcggcgcccccctgagcaaggaggtgggcgaggccgtggccaagaggttccacctgcccggcatcaggcagggctacggcctgaccgagaccaccagcgccatcctgatcacccccgagggcgacgacaagcccggcgccgtgggcaaggtggtgcccttcttcgaggccaaggtggtggacctggacaccggcaagaccctgggcgtgaaccagaggggcgagctgtgcgtgaggggccccatgatcatgagcggctacgtgaacaaccccgaggccaccaacgccctgatcgacaaggacggctggctgcacagcggcgacatcgcctactgggacgaggacgagcacttcttcatcgtggacaggctgaagagtctgatcaagtacaagggctaccaggtggcccccgccgagctggagagcatcctgctgcagcaccccaacatcttcgacgccggcgtggccggcctgcccgacgacgacgccggcgagctgcccgccgccgtggtggtgctggagcacggcaagaccatgaccgagaaggagatcgtggactacgtggccagccaggtgaccaccgccaagaagctgaggggcggcgtggtgttcgtggacgaggtgcccaagggcctgaccggcaagctggacgccaggaagatcagggagatcctgatcaaggccaagaagggcggcaagatcgccgtgtgatgagctcgctttcttgctgtccaatttctattaaaggttcctttgttccctaagtccaactactaaactgggggatattatgaagggccttgagcatctggattctgcctaataaaaaacatttattttcattgcgctcgctttcttgctgtccaatttctattaaaggttcctttgttccctaagtccaactactaaactgggggatattatgaagggccttgagcatctggattctgcctaataaaaaacatttattttcattgcaaaaaaaaaaaaaaaaaaaaaaaaaaaaaagaaaaaaaaaaaaaaaaaaaaaaaaaaaaaaaaaaaaaaaaaaaaaaaaaaaaaaaaaaaaaaaaaaaaaacgaagagcatcattgtcacatgtgagcaaaaggccagcaaaaggccaggaaccgtaaaaaggccgcgttgctggcgtttttccataggctccgcccccctgacgagcatcacaaaaatcgacgctcaagtcagaggtggcgaaacccgacaggactataaagataccaggcgtttccccctggaagctccctcgtgcgctctcctgttccgaccctgccgcttaccggatacctgtccgcctttctcccttcgggaagcgtggcgctttctcatagctcacgctgtaggtatctcagttcggtgtaggtcgttcgctccaagctgggctgtgtgcacgaaccccccgttcagcccgaccgctgcgccttatccggtaactatcgtcttgagtccaacccggtaagacacgacttatcgccactggcagcagccactggtaacaggattagcagagcgaggtatgtaggcggtgctacagagttcttgaagtggtggcctaactacggctacactagaagaacagtatttggtatctgcgctctgctgaagccagttaccttcggaaaaagagttggtagctcttgatccggcaaacaaaccaccgctggtagcggtggtttttttgtttgcaagcagcagattacgcgcagaaaaaaaggatctcaagaagatcctttgatcttttctacggggtctgacgctcagtggaacgaaaactcacgttaagggattttggtcatgagattatcaaaaaggatcttcacctagatccttttaaattaaaaatgaagttttaaatcaagcccaatctgaataatgttacaaccaattaaccaattctgattagaaaaactcatcgagcatcaaatgaaactgcaatttattcatatcaggattatcaataccatatttttgaaaaagccgtttctgtaatgaaggagaaaactcaccgaggcagttccataggatggcaagatcctggtatcggtctgcgattccgactcgtccaacatcaatacaacctattaatttcccctcgtcaaaaataaggttatcaagtgagaaatcaccatgagtgacgactgaatccggtgagaatggcaaaagtttatgcatttctttccagacttgttcaacaggccagccattacgctcgtcatcaaaatcactcgcatcaaccaaaccgttattcattcgtgattgcgcctgagcgagacgaaatacgcgatcgctgttaaaaggacaattacaaacaggaatcgaatgcaaccggcgcaggaacactgccagcgcatcaacaatattttcacctgaatcaggatattcttctaatacctggaatgctgtttttccggggatcgcagtggtgagtaaccatgcatcatcaggagtacggataaaatgcttgatggtcggaagaggcataaattccgtcagccagtttagtctgaccatctcatctgtaacatcattggcaacgctacctttgccatgtttcagaaacaactctggcgcatcgggcttcccatacaagcgatagattgtcgcacctgattgcccgacattatcgcgagcccatttatacccatataaatcagcatccatgttggaatttaatcgcggcctcgacgtttcccgttgaatatggctcataacaccccttgtattactgtttatgtaagcagacagttttattgttcatgatgatatatttttatcttgtgcaatgtaacatcagagattttgagacacgggccagagctgca

SEQ ID NO: 35 - DNA, 3943 bp, synthetic construct
  source 1..3943: mol_type = other DNA
tcgcgcgtttcggtgatgacggtgaaaacctctgacacatgcagctcccggacgtcattgtcgattaatacgactcactataaggaggcacagacaccaaggacagagacgctggctaggccgccctccccactgttaccaacgccaccgccaccatggaggacgccaagaacatcaagaagggccccgcccccttctaccccctggaggacggcaccgccggcgagcagctgcacaaggccatgaagaggtacgccctggtgcccggcaccatcgccttcaccgacgcccacatcgaggtggacatcacctacgccgagtacttcgagatgagcgtgaggctggccgaggccatgaagaggtacggcctgaacaccaaccacaggatcgtggtgtgcagcgagaacagcctgcagttcttcatgcccgtgctgggcgccctgttcatcggcgtggccgtggcccccgccaacgacatctacaacgagagggagctgctgaacagcatgggcatcagccagcccaccgtggtgttcgtgagcaagaagggcctgcagaagatcctgaacgtgcagaagaagctgcccatcatccagaagatcatcatcatggacagcaagaccgactaccagggcttccagagcatgtacaccttcgtgaccagccacctgccccccggcttcaacgagtacgacttcgtgcccgagagcttcgacagggacaagaccatcgccctgatcatgaacagcagcggcagcaccggcctgcccaagggcgtggccctgccccacaggaccgcctgcgtgaggttcagccacgccagggaccccatcttcggcaaccagatcatccccgacaccgccatcctgagcgtggtgcccttccaccacggcttcggcatgttcaccaccctgggctacctgatctgcggcttcagggtggtgctgatgtacaggttcgaggaggagctgttcctgaggagcctgcaggactacaagatccagagcgccctgctggtgcccaccctgttcagcttcttcgccaagagcaccctgatcgacaagtacgacctgagcaacctgcacgagatcgccagcggcggcgcccccctgagcaaggaggtgggcgaggccgtggccaagaggttccacctgcccggcatcaggcagggctacggcctgaccgagaccaccagcgccatcctgatcacccccgagggcgacgacaagcccggcgccgtgggcaaggtggtgcccttcttcgaggccaaggtggtggacctggacaccggcaagaccctgggcgtgaaccagaggggcgagctgtgcgtgaggggccccatgatcatgagcggctacgtgaacaaccccgaggccaccaacgccctgatcgacaaggacggctggctgcacagcggcgacatcgcctactgggacgaggacgagcacttcttcatcgtggacaggctgaagagtctgatcaagtacaagggctaccaggtggcccccgccgagctggagagcatcctgctgcagcaccccaacatcttcgacgccggcgtggccggcctgcccgacgacgacgccggcgagctgcccgccgccgtggtggtgctggagcacggcaagaccatgaccgagaaggagatcgtggactacgtggccagccaggtgaccaccgccaagaagctgaggggcggcgtggtgttcgtggacgaggtgcccaagggcctgaccggcaagctggacgccaggaagatcagggagatcctgatcaaggccaagaagggcggcaagatcgccgtgtgatgagctcgctttcttgctgtccaatttctattaaaggttcctttgttccctaagtccaactactaaactgggggatattatgaagggccttgagcatctggattctgcctaataaaaaacatttattttcattgcgctcgctttcttgctgtccaatttctattaaaggttcctttgttccctaagtccaactactaaactgggggatattatgaagggccttgagcatctggattctgcctaataaaaaacatttattttcattgcaaaaaaaaaaaaaaaaaaaaaaaaaaaaaagaaaaaaaaaaaaaaaaaaaaaaaaaaaaaaaaaaaaaaaaaaaaaaaaaaaaaaaaaaaaaaaaaaaaaacgaagagcatcattgtcacatgtgagcaaaaggccagcaaaaggccaggaaccgtaaaaaggccgcgttgctggcgtttttccataggctccgcccccctgacgagcatcacaaaaatcgacgctcaagtcagaggtggcgaaacccgacaggactataaagataccaggcgtttccccctggaagctccctcgtgcgctctcctgttccgaccctgccgcttaccggatacctgtccgcctttctcccttcgggaagcgtggcgctttctcatagctcacgctgtaggtatctcagttcggtgtaggtcgttcgctccaagctgggctgtgtgcacgaaccccccgttcagcccgaccgctgcgccttatccggtaactatcgtcttgagtccaacccggtaagacacgacttatcgccactggcagcagccactggtaacaggattagcagagcgaggtatgtaggcggtgctacagagttcttgaagtggtggcctaactacggctacactagaagaacagtatttggtatctgcgctctgctgaagccagttaccttcggaaaaagagttggtagctcttgatccggcaaacaaaccaccgctggtagcggtggtttttttgtttgcaagcagcagattacgcgcagaaaaaaaggatctcaagaagatcctttgatcttttctacggggtctgacgctcagtggaacgaaaactcacgttaagggattttggtcatgagattatcaaaaaggatcttcacctagatccttttaaattaaaaatgaagttttaaatcaagcccaatctgaataatgttacaaccaattaaccaattctgattagaaaaactcatcgagcatcaaatgaaactgcaatttattcatatcaggattatcaataccatatttttgaaaaagccgtttctgtaatgaaggagaaaactcaccgaggcagttccataggatggcaagatcctggtatcggtctgcgattccgactcgtccaacatcaatacaacctattaatttcccctcgtcaaaaataaggttatcaagtgagaaatcaccatgagtgacgactgaatccggtgagaatggcaaaagtttatgcatttctttccagacttgttcaacaggccagccattacgctcgtcatcaaaatcactcgcatcaaccaaaccgttattcattcgtgattgcgcctgagcgagacgaaatacgcgatcgctgttaaaaggacaattacaaacaggaatcgaatgcaaccggcgcaggaacactgccagcgcatcaacaatattttcacctgaatcaggatattcttctaatacctggaatgctgtttttccggggatcgcagtggtgagtaaccatgcatcatcaggagtacggataaaatgcttgatggtcggaagaggcataaattccgtcagccagtttagtctgaccatctcatctgtaacatcattggcaacgctacctttgccatgtttcagaaacaactctggcgcatcgggcttcccatacaagcgatagattgtcgcacctgattgcccgacattatcgcgagcccatttatacccatataaatcagcatccatgttggaatttaatcgcggcctcgacgtttcccgttgaatatggctcataacaccccttgtattactgtttatgtaagcagacagttttattgttcatgatgatatatttttatcttgtgcaatgtaacatcagagattttgagacacgggccagagctgca

SEQ ID NO: 36 - DNA, 3785 bp, synthetic construct
  source 1..3785: mol_type = other DNA
tcgcgcgtttcggtgatgacggtgaaaacctctgacacatgcagctcccggacgtcattgtcgattaatacgactcactataaggaaataagagagaaaagaagagtaagaagaaatataagaccccggcgccgccaccatggaggacgccaagaacatcaagaagggccccgcccccttctaccccctggaggacggcaccgccggcgagcagctgcacaaggccatgaagaggtacgccctggtgcccggcaccatcgccttcaccgacgcccacatcgaggtggacatcacctacgccgagtacttcgagatgagcgtgaggctggccgaggccatgaagaggtacggcctgaacaccaaccacaggatcgtggtgtgcagcgagaacagcctgcagttcttcatgcccgtgctgggcgccctgttcatcggcgtggccgtggcccccgccaacgacatctacaacgagagggagctgctgaacagcatgggcatcagccagcccaccgtggtgttcgtgagcaagaagggcctgcagaagatcctgaacgtgcagaagaagctgcccatcatccagaagatcatcatcatggacagcaagaccgactaccagggcttccagagcatgtacaccttcgtgaccagccacctgccccccggcttcaacgagtacgacttcgtgcccgagagcttcgacagggacaagaccatcgccctgatcatgaacagcagcggcagcaccggcctgcccaagggcgtggccctgccccacaggaccgcctgcgtgaggttcagccacgccagggaccccatcttcggcaaccagatcatccccgacaccgccatcctgagcgtggtgcccttccaccacggcttcggcatgttcaccaccctgggctacctgatctgcggcttcagggtggtgctgatgtacaggttcgaggaggagctgttcctgaggagcctgcaggactacaagatccagagcgccctgctggtgcccaccctgttcagcttcttcgccaagagcaccctgatcgacaagtacgacctgagcaacctgcacgagatcgccagcggcggcgcccccctgagcaaggaggtgggcgaggccgtggccaagaggttccacctgcccggcatcaggcagggctacggcctgaccgagaccaccagcgccatcctgatcacccccgagggcgacgacaagcccggcgccgtgggcaaggtggtgcccttcttcgaggccaaggtggtggacctggacaccggcaagaccctgggcgtgaaccagaggggcgagctgtgcgtgaggggccccatgatcatgagcggctacgtgaacaaccccgaggccaccaacgccctgatcgacaaggacggctggctgcacagcggcgacatcgcctactgggacgaggacgagcacttcttcatcgtggacaggctgaagagtctgatcaagtacaagggctaccaggtggcccccgccgagctggagagcatcctgctgcagcaccccaacatcttcgacgccggcgtggccggcctgcccgacgacgacgccggcgagctgcccgccgccgtggtggtgctggagcacggcaagaccatgaccgagaaggagatcgtggactacgtggccagccaggtgaccaccgccaagaagctgaggggcggcgtggtgttcgtggacgaggtgcccaagggcctgaccggcaagctggacgccaggaagatcagggagatcctgatcaaggccaagaagggcggcaagatcgccgtgtgataataggctggagcctcggtggcctagcttcttgccccttgggcctccccccagcccctcctccccttcctgcacccgtacccccgtggtctttgaataaagtctgagtgggcggcaaaaaaaaaaaaaaaaaaaaaaaaaaaaaagcatatgactaaaaaaaaaaaaaaaaaaaaaaaaaaaaaaaaaaaaaaaaaaaaaaaaaaaaaaaaaaaaaaaaaaaaaagcggccgcatcattgtcacatgtgagcaaaaggccagcaaaaggccaggaaccgtaaaaaggccgcgttgctggcgtttttccataggctccgcccccctgacgagcatcacaaaaatcgacgctcaagtcagaggtggcgaaacccgacaggactataaagataccaggcgtttccccctggaagctccctcgtgcgctctcctgttccgaccctgccgcttaccggatacctgtccgcctttctcccttcgggaagcgtggcgctttctcatagctcacgctgtaggtatctcagttcggtgtaggtcgttcgctccaagctgggctgtgtgcacgaaccccccgttcagcccgaccgctgcgccttatccggtaactatcgtcttgagtccaacccggtaagacacgacttatcgccactggcagcagccactggtaacaggattagcagagcgaggtatgtaggcggtgctacagagttcttgaagtggtggcctaactacggctacactagaagaacagtatttggtatctgcgctctgctgaagccagttaccttcggaaaaagagttggtagctcttgatccggcaaacaaaccaccgctggtagcggtggtttttttgtttgcaagcagcagattacgcgcagaaaaaaaggatctcaagaagatcctttgatcttttctacggggtctgacgctcagtggaacgaaaactcacgttaagggattttggtcatgagattatcaaaaaggatcttcacctagatccttttaaattaaaaatgaagttttaaatcaagcccaatctgaataatgttacaaccaattaaccaattctgattagaaaaactcatcgagcatcaaatgaaactgcaatttattcatatcaggattatcaataccatatttttgaaaaagccgtttctgtaatgaaggagaaaactcaccgaggcagttccataggatggcaagatcctggtatcggtctgcgattccgactcgtccaacatcaatacaacctattaatttcccctcgtcaaaaataaggttatcaagtgagaaatcaccatgagtgacgactgaatccggtgagaatggcaaaagtttatgcatttctttccagacttgttcaacaggccagccattacgctcgtcatcaaaatcactcgcatcaaccaaaccgttattcattcgtgattgcgcctgagcgagacgaaatacgcgatcgctgttaaaaggacaattacaaacaggaatcgaatgcaaccggcgcaggaacactgccagcgcatcaacaatattttcacctgaatcaggatattcttctaatacctggaatgctgtttttccggggatcgcagtggtgagtaaccatgcatcatcaggagtacggataaaatgcttgatggtcggaagaggcataaattccgtcagccagtttagtctgaccatctcatctgtaacatcattggcaacgctacctttgccatgtttcagaaacaactctggcgcatcgggcttcccatacaagcgatagattgtcgcacctgattgcccgacattatcgcgagcccatttatacccatataaatcagcatccatgttggaatttaatcgcggcctcgacgtttcccgttgaatatggctcataacaccccttgtattactgtttatgtaagcagacagttttattgttcatgatgatatatttttatcttgtgcaatgtaacatcagagattttgagacacgggccagagctgca

SEQ ID NO: 37 - DNA, 3764 bp, synthetic construct
  source 1..3764: mol_type = other DNA
tcgcgcgtttcggtgatgacggtgaaaacctctgacacatgcagctcccggacgtcattgtcgattaatacgactcactataaggaaataagagagaaaagaagagtaagaagaaatataagagccaccatggaagacgccaagaacattaagaaggggccggccccgttctacccgttggaagacgggaccgccggggaacagttgcacaaggccatgaagagatacgccttggtgccggggaccattgccttcaccgacgcccacattgaagtggacattacctacgccgaatacttcgaaatgtcggtgagattggccgaagccatgaagagatacgggttgaacaccaaccacagaattgtggtgtgctcggaaaactcgttgcagttcttcatgccggtgttgggggccttgttcattggggtggccgtggccccggccaacgacatttacaacgaaagagaattgttgaactcgatggggatttcgcagccgaccgtggtgttcgtgtcgaagaaggggttgcagaagattttgaacgtgcagaagaagttgccgattattcagaagattattattatggactcgaagaccgactaccaggggttccagtcgatgtacaccttcgtgacctcgcacttgccgccggggttcaacgaatacgacttcgtgccggaatcgttcgacagagacaagaccattgccttgattatgaactcgtcggggtcgaccgggttgccgaagggggtggccttgccgcacagaaccgcctgcgtgagattctcgcacgccagagacccgattttcgggaaccagattattccggacaccgccattttgtcggtggtgccgttccaccacgggttcgggatgttcaccaccttggggtacttgatttgcgggttcagagtggtgttgatgtacagattcgaagaagaattgttcttgagatcgttgcaggactacaagattcagtcggccttgttggtgccgaccttgttctcgttcttcgccaagtcgaccttgattgacaagtacgacttgtcgaacttgcacgaaattgcctcggggggggccccgttgtcgaaggaagtgggggaagccgtggccaagagattccacttgccggggattagacaggggtacgggttgaccgaaaccacctcggccattttgattaccccggaaggggacgacaagccgggggccgtggggaaggtggtgccgttcttcgaagccaaggtggtggacttggacaccgggaagaccttgggggtgaaccagagaggggaattgtgcgtgagagggccgatgattatgtcggggtacgtgaacaacccggaagccaccaacgccttgattgacaaggacgggtggttgcactcgggggacattgcctactgggacgaagacgaacacttcttcattgtggacagattgaagtcgttgattaagtacaaggggtaccaggtggccccggccgaattggaatcgattttgttgcagcacccgaacattttcgacgccggggtggccgggttgccggacgacgacgccggggaattgccggccgccgtggtggtgttggaacacgggaagaccatgaccgaaaaggaaattgtggactacgtggcctcgcaggtgaccaccgccaagaagttgagagggggggtggtgttcgtggacgaagtgccgaaggggttgaccgggaagttggacgccagaaagattagagaaattttgattaaggccaagaagggggggaagattgccgtgtgataataggctggagcctcggtggccatgcttcttgccccttgggcctccccccagcccctcctccccttcctgcacccgtacccccgtggtctttgaataaagtctgagtgggcggaaaaaaaaaaaaaaaaaaaaaaaaaaaaaaaaaaaaaaaaaaaaaaaaaaaaaaaaaaaaaaaaaaaaaaaaaaaaaaaaaaaaaaaaaaaaaaaaaaaacgaagagcatcattgtcacatgtgagcaaaaggccagcaaaaggccaggaaccgtaaaaaggccgcgttgctggcgtttttccataggctccgcccccctgacgagcatcacaaaaatcgacgctcaagtcagaggtggcgaaacccgacaggactataaagataccaggcgtttccccctggaagctccctcgtgcgctctcctgttccgaccctgccgcttaccggatacctgtccgcctttctcccttcgggaagcgtggcgctttctcatagctcacgctgtaggtatctcagttcggtgtaggtcgttcgctccaagctgggctgtgtgcacgaaccccccgttcagcccgaccgctgcgccttatccggtaactatcgtcttgagtccaacccggtaagacacgacttatcgccactggcagcagccactggtaacaggattagcagagcgaggtatgtaggcggtgctacagagttcttgaagtggtggcctaactacggctacactagaagaacagtatttggtatctgcgctctgctgaagccagttaccttcggaaaaagagttggtagctcttgatccggcaaacaaaccaccgctggtagcggtggtttttttgtttgcaagcagcagattacgcgcagaaaaaaaggatctcaagaagatcctttgatcttttctacggggtctgacgctcagtggaacgaaaactcacgttaagggattttggtcatgagattatcaaaaaggatcttcacctagatccttttaaattaaaaatgaagttttaaatcaagcccaatctgaataatgttacaaccaattaaccaattctgattagaaaaactcatcgagcatcaaatgaaactgcaatttattcatatcaggattatcaataccatatttttgaaaaagccgtttctgtaatgaaggagaaaactcaccgaggcagttccataggatggcaagatcctggtatcggtctgcgattccgactcgtccaacatcaatacaacctattaatttcccctcgtcaaaaataaggttatcaagtgagaaatcaccatgagtgacgactgaatccggtgagaatggcaaaagtttatgcatttctttccagacttgttcaacaggccagccattacgctcgtcatcaaaatcactcgcatcaaccaaaccgttattcattcgtgattgcgcctgagcgagacgaaatacgcgatcgctgttaaaaggacaattacaaacaggaatcgaatgcaaccggcgcaggaacactgccagcgcatcaacaatattttcacctgaatcaggatattcttctaatacctggaatgctgtttttccggggatcgcagtggtgagtaaccatgcatcatcaggagtacggataaaatgcttgatggtcggaagaggcataaattccgtcagccagtttagtctgaccatctcatctgtaacatcattggcaacgctacctttgccatgtttcagaaacaactctggcgcatcgggcttcccatacaagcgatagattgtcgcacctgattgcccgacattatcgcgagcccatttatacccatataaatcagcatccatgttggaatttaatcgcggcctcgacgtttcccgttgaatatggctcataacaccccttgtattactgtttatgtaagcagacagttttattgttcatgatgatatatttttatcttgtgcaatgtaacatcagagattttgagacacgggccagagctgca

SEQ ID NO: 38 - DNA, 3752 bp, synthetic construct
  source 1..3752: mol_type = other DNA
tcgcgcgtttcggtgatgacggtgaaaacctctgacacatgcagctcccggacgtcattgtcgattaatacgactcactataaggaaataagagagaaaagaagagtaagaagaaatataagagccaccatggaggacgccaagaacatcaagaagggccccgcccccttctaccccctggaggacggcaccgccggcgagcagctgcacaaggccatgaagcggtacgccctggtgcccggcaccatcgccttcaccgacgcccacatcgaggtggacatcacctacgccgagtacttcgagatgagcgtgcggctggccgaggccatgaagcggtacggcctgaacaccaaccaccggatcgtggtgtgcagcgagaacagcctgcagttcttcatgcccgtgctgggcgccctgttcatcggcgtggccgtggcccccgccaacgacatctacaacgagcgggagctgctgaacagcatgggcatcagccagcccaccgtggtgttcgtgagcaagaagggcctgcagaagatcctgaacgtgcagaagaagctgcccatcatccagaagatcatcatcatggacagcaagaccgactaccagggcttccagagcatgtacaccttcgtgaccagccacctgccccccggcttcaacgagtacgacttcgtgcccgagagcttcgaccgggacaagaccatcgccctgatcatgaacagcagcggcagcaccggcctgcccaagggcgtggccctgccccaccggaccgcctgcgtgcggttcagccacgcccgggaccccatcttcggcaaccagatcatccccgacaccgccatcctgagcgtggtgcccttccaccacggcttcggcatgttcaccaccctgggctacctgatctgcggcttccgggtggtgctgatgtaccggttcgaggaggagctgttcctgcggagcctgcaggactacaagatccagagcgccctgctggtgcccaccctgttcagcttcttcgccaagagcaccctgatcgacaagtacgacctgagcaacctgcacgagatcgccagcggcggcgcccccctgagcaaggaggtgggcgaggccgtggccaagcggttccacctgcccggcatccggcagggctacggcctgaccgagaccaccagcgccatcctgatcacccccgagggcgacgacaagcccggcgccgtgggcaaggtggtgcccttcttcgaggccaaggtggtggacctggacaccggcaagaccctgggcgtgaaccagcggggcgagctgtgcgtgcggggccccatgatcatgagcggctacgtgaacaaccccgaggccaccaacgccctgatcgacaaggacggctggctgcacagcggcgacatcgcctactgggacgaggacgagcacttcttcatcgtggaccggctgaagagcctgatcaagtacaagggctaccaggtggcccccgccgagctggagagcatcctgctgcagcaccccaacatcttcgacgccggcgtggccggcctgcccgacgacgacgccggcgagctgcccgccgccgtggtggtgctggagcacggcaagaccatgaccgagaaggagatcgtggactacgtggccagccaggtgaccaccgccaagaagctgcggggcggcgtggtgttcgtggacgaggtgcccaagggcctgaccggcaagctggacgcccggaagatccgggagatcctgatcaaggccaagaagggcggcaagatcgccgtgtgattaattaagctgccttctgcggggcttgccttctggccatgcccttcttctctcccttgcacctgtacctcttggtctttgaataaagcctgagtaggaagaaaaaaaaaaaaaaaaaaaaaaaaaaaaaaaaaaaaaaaaaaaaaaaaaaaaaaaaaaaaaaaaaaaaaaaaaaaaaaaaaaaaaaaaaaaaaaaaaaaaaagcggccgcatcattgtcacatgtgagcaaaaggccagcaaaaggccaggaaccgtaaaaaggccgcgttgctggcgtttttccataggctccgcccccctgacgagcatcacaaaaatcgacgctcaagtcagaggtggcgaaacccgacaggactataaagataccaggcgtttccccctggaagctccctcgtgcgctctcctgttccgaccctgccgcttaccggatacctgtccgcctttctcccttcgggaagcgtggcgctttctcatagctcacgctgtaggtatctcagttcggtgtaggtcgttcgctccaagctgggctgtgtgcacgaaccccccgttcagcccgaccgctgcgccttatccggtaactatcgtcttgagtccaacccggtaagacacgacttatcgccactggcagcagccactggtaacaggattagcagagcgaggtatgtaggcggtgctacagagttcttgaagtggtggcctaactacggctacactagaagaacagtatttggtatctgcgctctgctgaagccagttaccttcggaaaaagagttggtagctcttgatccggcaaacaaaccaccgctggtagcggtggtttttttgtttgcaagcagcagattacgcgcagaaaaaaaggatctcaagaagatcctttgatcttttctacggggtctgacgctcagtggaacgaaaactcacgttaagggattttggtcatgagattatcaaaaaggatcttcacctagatccttttaaattaaaaatgaagttttaaatcaagcccaatctgaataatgttacaaccaattaaccaattctgattagaaaaactcatcgagcatcaaatgaaactgcaatttattcatatcaggattatcaataccatatttttgaaaaagccgtttctgtaatgaaggagaaaactcaccgaggcagttccataggatggcaagatcctggtatcggtctgcgattccgactcgtccaacatcaatacaacctattaatttcccctcgtcaaaaataaggttatcaagtgagaaatcaccatgagtgacgactgaatccggtgagaatggcaaaagtttatgcatttctttccagacttgttcaacaggccagccattacgctcgtcatcaaaatcactcgcatcaaccaaaccgttattcattcgtgattgcgcctgagcgagacgaaatacgcgatcgctgttaaaaggacaattacaaacaggaatcgaatgcaaccggcgcaggaacactgccagcgcatcaacaatattttcacctgaatcaggatattcttctaatacctggaatgctgtttttccggggatcgcagtggtgagtaaccatgcatcatcaggagtacggataaaatgcttgatggtcggaagaggcataaattccgtcagccagtttagtctgaccatctcatctgtaacatcattggcaacgctacctttgccatgtttcagaaacaactctggcgcatcgggcttcccatacaagcgatagattgtcgcacctgattgcccgacattatcgcgagcccatttatacccatataaatcagcatccatgttggaatttaatcgcggcctcgacgtttcccgttgaatatggctcataacaccccttgtattactgtttatgtaagcagacagttttattgttcatgatgatatatttttatcttgtgcaatgtaacatcagagattttgagacacgggccagagctgca

SEQ ID NO: 39 - RNA, 101 nt, synthetic construct
  source 1..101: mol_type = other RNA
aaaaaaaaaaaaaaaaaaaaaaaaaaaaaagaaaaaaaaaaaaaaaaaaaaaaaaaaaaaaaaaaaaaaaaaaaaaaaaaaaaaaaaaaaaaaaaaaaaaa